European Patent Specification EP 3 737 755 B1, published August 28, 2024. Title: COMPOSITIONS AND METHODS FOR TEMPLATE-FREE GEOMETRIC ENZYMATIC NUCLEIC ACID SYNTHESIS. Applicant: Camena Bioscience Limited Fraser, Andrew G Stemple, Derek L Mankowska, Sylwia A. The sequence listing filed with the application follows.

SEQUENCE LISTING (104 sequences)

SEQ ID NO: 1 - DNA, 210 bp, Aequorea victoria
tacacacgaataaaagataacaaagatgagtaaaggagaagaacttttcactggagttgtcccaattcttgttgaattagatggcgatgttaatgggcaaaaattctctgtcagtggagagggtgaaggtgatgcaacatacggaaaacttacccttaaatttatttgcactactgggaagctacctgttccatggccaacacttgtcac

SEQ ID NO: 2 - DNA, 21 bp, Artificial Sequence
  N-mer
tacacacgaataaaagataac

SEQ ID NO: 3 - DNA, 21 bp, Artificial Sequence
  N-mer
acttttcactggagttgtccc

SEQ ID NO: 4 - DNA, 21 bp, Artificial Sequence
  N-mer
cgatgttaatgggcaaaaatt

SEQ ID NO: 5 - DNA, 21 bp, Artificial Sequence
  N-mer
aggtgatgcaacatacggaaa

SEQ ID NO: 6 - DNA, 21 bp, Artificial Sequence
  N-mer
aaagatgagtaaaggagaaga

SEQ ID NO: 7 - DNA, 21 bp, Artificial Sequence
  N-mer
aattcttgttgaattagatgg

SEQ ID NO: 8 - DNA, 21 bp, Artificial Sequence
  N-mer
ctctgtcagtggagagggtga

SEQ ID NO: 9 - DNA, 21 bp, Artificial Sequence
  N-mer
acttacccttaaatttatttg

SEQ ID NO: 10 - DNA, 18 bp, Artificial Sequence
  T7 promoter sequence
ctatagtgagtcgtatta

SEQ ID NO: 11 - DNA, 39 bp, Artificial Sequence
  Anchor primer
ctatagtgagtcgtattaccgtagtgctgcgtcgagtgt

SEQ ID NO: 12 - DNA, 41 bp, Artificial Sequence
  Anchor primer
  misc_feature (1)..(1): ribonucleotide
  misc_feature (2)..(41): deoxyribonucleotide
uccattgtgagtcttatttccgtagtgctgcgtcgagtgtc

SEQ ID NO: 13 - DNA, 12 bp, Artificial Sequence
  N-mer
  misc_feature (1)..(11): deoxyribonucleotide
  misc_feature (12)..(12): ribonucleotide
ccgtccttcacc

SEQ ID NO: 14 - DNA, 12 bp, Artificial Sequence
  N-mer
  misc_feature (1)..(11): deoxyribonucleotide
  misc_feature (12)..(12): ribonucleotide
gaactactggac

SEQ ID NO: 15 - DNA, 12 bp, Artificial Sequence
  N-mer
  misc_feature (1)..(11): deoxyribonucleotide
  misc_feature (12)..(12): ribonucleotide
ctcaacagtagc

SEQ ID NO: 16 - DNA, 15 bp, Artificial Sequence
  N-mer
  misc_feature (1)..(11): deoxyribonucleotide
  misc_feature (12)..(12): ribonucleotide
ggagctcacactcta

SEQ ID NO: 17 - DNA, 35 bp, Artificial Sequence
  Anchor primer
tggaattctcgggtgccaaggatgttttttttttt

SEQ ID NO: 18 - DNA, 30 bp, Artificial Sequence
  Anchor primer
  misc_feature (1)..(29): deoxyribonucleotide
  misc_feature (30)..(30): ribonucleotide
ttttttttttgtagtgctgcgtgctcttca

SEQ ID NO: 19 - RNA, 12 nt, Artificial Sequence
  N-mer
ggugaaggacgg

SEQ ID NO: 20 - DNA, 19 bp, Artificial Sequence
  Short reverse complementary oligonucleotide
gaagagcacgcagcactac

SEQ ID NO: 21 - DNA, 12 bp, Artificial Sequence
  N-mer
  misc_feature (1)..(11): deoxyribonucleotide
  misc_feature (12)..(12): ribonucleotide
ccgtccttcacc

SEQ ID NO: 22 - RNA, 12 nt, Artificial Sequence
  N-mer
gagugugagcuc

SEQ ID NO: 23 - DNA, 59 bp, Artificial Sequence
  N-mer
tacacgacgctctctgaagacactcgatccctacacgacgccgtccgttctacctcttt

SEQ ID NO: 24 - DNA, 40 bp, Artificial Sequence
  N-mer
gacacatgaaagcttgaattcacggcatatgagtccatgg

SEQ ID NO: 25 - DNA, 30 bp, Artificial Sequence
  N-mer
  misc_feature (1)..(29): deoxyribonucleotide
  misc_feature (30)..(30): ribonucleotide
ttttttttttcttccgatctgagtccagcg

SEQ ID NO: 26 - RNA, 26 nt, Artificial Sequence
  N-mer
guucagaguucuacaguccgacgauc

SEQ ID NO: 27 - DNA, 31 bp, Artificial Sequence
  N-mer
  misc_feature (23)..(23): fluorescein-labeled base
aagtagcgaactactggacccgtccttcacc

SEQ ID NO: 28 - DNA, 31 bp, Artificial Sequence
  N-mer
  misc_feature (23)..(23): fluorescein-labeled base
cagtagcgaactactggacccgtccttcacc

SEQ ID NO: 29 - DNA, 31 bp, Artificial Sequence
  N-mer
  misc_feature (23)..(23): fluorescein-labeled base
gagtagcgaactactggacccgtccttcacc

SEQ ID NO: 30 - DNA, 31 bp, Artificial Sequence
  N-mer
  misc_feature (23)..(23): fluorescein-labeled base
tagtagcgaactactggacccgtccttcacc

SEQ ID NO: 31 - DNA, 18 bp, Artificial Sequence
  N-mer
actagttacggagctcac

SEQ ID NO: 32 - DNA, 18 bp, Artificial Sequence
  N-mer
tgaatgaaatggtgaagg

SEQ ID NO: 33 - DNA, 17 bp, Artificial Sequence
  N-mer
cgctttaggttaagact

SEQ ID NO: 34 - DNA, 20 bp, Artificial Sequence
  N-mer
  misc_feature (1)..(19): deoxyribonucleotide
  misc_feature (20)..(20): ribonucleotide
ggagctcacactctactcaa

SEQ ID NO: 35 - DNA, 20 bp, Artificial Sequence
  N-mer
  misc_feature (1)..(19): deoxyribonucleotide
  misc_feature (20)..(20): ribonucleotide
ggagctcacactctactcac

SEQ ID NO: 36 - DNA, 20 bp, Artificial Sequence
  N-mer
  misc_feature (1)..(19): deoxyribonucleotide
  misc_feature (20)..(20): ribonucleotide
ggagctcacactctactcag

SEQ ID NO: 37 - DNA, 20 bp, Artificial Sequence
  N-mer
  misc_feature (1)..(19): deoxyribonucleotide
  misc_feature (20)..(20): ribonucleotide
ggagctcacactctactcat

SEQ ID NO: 38 - DNA, 58 bp, Artificial Sequence
  Anchor primer
ccatggactcatatgccgtgaattcaagctttcatgtgtcttcatagtccgtcgtgta

SEQ ID NO: 39 - RNA, 20 nt, Artificial Sequence
  N-mer
aguucugcagucugcagaaa

SEQ ID NO: 40 - DNA, 54 bp, Artificial Sequence
  Anchor primer
ctctctctctctctctctctctctctctctcccttcctttctctgagtctgtag

SEQ ID NO: 41 - DNA, 24 bp, Artificial Sequence
  Short reverse complementary oligonucleotide
gggaaggaaagagactcagacatc

SEQ ID NO: 42 - DNA, 52 bp, Artificial Sequence
  Anchor primer
cttaagactcgatatccctgcaggctctctctctctctctctctctctctct

SEQ ID NO: 43 - DNA, 24 bp, Artificial Sequence
  Short reverse complementary oligonucleotide
gaattctgagctatagggacgtcc

SEQ ID NO: 44 - DNA, 55 bp, Artificial Sequence
  Anchor primer
  misc_feature (1)..(54): deoxyribonucleotide
  misc_feature (55)..(55): ribonucleotide
ctctctctctctctctctctctctctctctctctctctctctctctctctctctu

SEQ ID NO: 45 - DNA, 47 bp, Artificial Sequence
  Anchor primer
  modified_base (2)..(2): I
  misc_feature (2)..(2): n is a, c, g, or t
anctctctctctctctctcctctctctctctctctctctctctctct

SEQ ID NO: 46 - DNA, 922 bp, Aequorea victoria
tacacacgaataaaagataacaaagatgagtaaaggagaagaacttttcactggagttgtcccaattcttgttgaattagatggcgatgttaatgggcaaaaattctctgtcagtggagagggtgaaggtgatgcaacatacggaaaacttacccttaaatttatttgcactactgggaagctacctgttccatggccaacacttgtcactactttctcttatggtgttcaatgcttttcaagatacccagatcatatgaaacagcatgactttttcaagagtgccatgcccgaaggttatgtacaggaaagaactatattttacaaagatgacgggaactacaagacacgtgctgaagtcaagtttgaaggtgatacccttgttaatagaatcgagttaaaaggtattgattttaaagaagatggaaacattcttggacacaaaatggaatacaactataactcacataatgtatacatcatggcagacaaaccaaagaatggaatcaaagttaacttcaaaattagacacaacattaaagatggaagcgttcaattagcagaccattatcaacaaaatactccaattggcgatggccctgtccttttaccagacaaccattacctgtccacacaatctgccctttccaaagatcccaacgaaaagagagatcacatgatccttcttgagtttgtaacagctgctgggattacacatggcatggatgaactatacaaataaatgtccagacttccaattgacactaaagtgtccgaacaattactaaattctcagggttcctggttaaattcaggctgagactttatttatatatttatagattcattaaaattttatgaataatttattgatgttattaataggggctattttcttattaaataggctactggagtgtat

SEQ ID NO: 47 - DNA, 21 bp, Artificial Sequence
  N-mer
tacacacgaataaaagataac

SEQ ID NO: 48 - DNA, 21 bp, Artificial Sequence
  N-mer
acttttcactggagttgtccc

SEQ ID NO: 49 - DNA, 21 bp, Artificial Sequence
  N-mer
cgatgttaatgggcaaaaatt

SEQ ID NO: 50 - DNA, 21 bp, Artificial Sequence
  N-mer
aggtgatgcaacatacggaaa

SEQ ID NO: 51 - DNA, 21 bp, Artificial Sequence
  N-mer
cactactgggaagctacctgt

SEQ ID NO: 52 - DNA, 21 bp, Artificial Sequence
  N-mer
tactttctcttatggtgttca

SEQ ID NO: 53 - DNA, 21 bp, Artificial Sequence
  N-mer
tcatatgaaacagcatgactt

SEQ ID NO: 54 - DNA, 21 bp, Artificial Sequence
  N-mer
aggttatgtacaggaaagaac

SEQ ID NO: 55 - DNA, 21 bp, Artificial Sequence
  N-mer
gaactacaagacacgtgctga

SEQ ID NO: 56 - DNA, 21 bp, Artificial Sequence
  N-mer
ccttgttaatagaatcgagtt

SEQ ID NO: 57 - DNA, 21 bp, Artificial Sequence
  N-mer
agatggaaacattcttggaca

SEQ ID NO: 58 - DNA, 21 bp, Artificial Sequence
  N-mer
ctcacataatgtatacatcat

SEQ ID NO: 59 - DNA, 21 bp, Artificial Sequence
  N-mer
aatcaaagttaacttcaaaat

SEQ ID NO: 60 - DNA, 21 bp, Artificial Sequence
  N-mer
aagcgttcaattagcagacca

SEQ ID NO: 61 - DNA, 21 bp, Artificial Sequence
  N-mer
tggcgatggccctgtcctttt

SEQ ID NO: 62 - DNA, 21 bp, Artificial Sequence
  N-mer
cacacaatctgccctttccaa

SEQ ID NO: 63 - DNA, 21 bp, Artificial Sequence
  N-mer
tcacatgatccttcttgagtt

SEQ ID NO: 64 - DNA, 21 bp, Artificial Sequence
  N-mer
acatggcatggatgaactata

SEQ ID NO: 65 - DNA, 21 bp, Artificial Sequence
  N-mer
aattgacactaaagtgtccga

SEQ ID NO: 66 - DNA, 21 bp, Artificial Sequence
  N-mer
ttcctggttaaattcaggctg

SEQ ID NO: 67 - DNA, 21 bp, Artificial Sequence
  N-mer
agattcattaaaattttatga

SEQ ID NO: 68 - DNA, 21 bp, Artificial Sequence
  N-mer
taggggctattttcttattaa

SEQ ID NO: 69 - DNA, 21 bp, Artificial Sequence
  N-mer
aaagatgagtaaaggagaaga

SEQ ID NO: 70 - DNA, 21 bp, Artificial Sequence
  N-mer
aattcttgttgaattagatgg

SEQ ID NO: 71 - DNA, 21 bp, Artificial Sequence
  N-mer
ctctgtcagtggagagggtga

SEQ ID NO: 72 - DNA, 21 bp, Artificial Sequence
  N-mer
acttacccttaaatttatttg

SEQ ID NO: 73 - DNA, 21 bp, Artificial Sequence
  N-mer
tccatggccaacacttgtcac

SEQ ID NO: 74 - DNA, 21 bp, Artificial Sequence
  N-mer
atgcttttcaagatacccaga

SEQ ID NO: 75 - DNA, 21 bp, Artificial Sequence
  N-mer
tttcaagagtgccatgcccga

SEQ ID NO: 76 - DNA, 21 bp, Artificial Sequence
  N-mer
tatattttacaaagatgacgg

SEQ ID NO: 77 - DNA, 21 bp, Artificial Sequence
  N-mer
agtcaagtttgaaggtgatac

SEQ ID NO: 78 - DNA, 21 bp, Artificial Sequence
  N-mer
aaaaggtattgattttaaaga

SEQ ID NO: 79 - DNA, 21 bp, Artificial Sequence
  N-mer
caaaatggaatacaactataa

SEQ ID NO: 80 - DNA, 21 bp, Artificial Sequence
  N-mer
ggcagacaaaccaaagaatgg

SEQ ID NO: 81 - DNA, 21 bp, Artificial Sequence
  N-mer
tagacacaacattaaagatgg

SEQ ID NO: 82 - DNA, 21 bp, Artificial Sequence
  N-mer
ttatcaacaaaatactccaat

SEQ ID NO: 83 - DNA, 21 bp, Artificial Sequence
  N-mer
accagacaaccattacctgtc

SEQ ID NO: 84 - DNA, 21 bp, Artificial Sequence
  N-mer
agatcccaacgaaaagagaga

SEQ ID NO: 85 - DNA, 21 bp, Artificial Sequence
  N-mer
tgtaacagctgctgggattac

SEQ ID NO: 86 - DNA, 21 bp, Artificial Sequence
  N-mer
caaataaatgtccagacttcc

SEQ ID NO: 87 - DNA, 21 bp, Artificial Sequence
  N-mer
acaattactaaattctcaggg

SEQ ID NO: 88 - DNA, 21 bp, Artificial Sequence
  N-mer
agactttatttatatatttat

SEQ ID NO: 89 - DNA, 21 bp, Artificial Sequence
  N-mer
ataatttattgatgttattaa

SEQ ID NO: 90 - DNA, 19 bp, Artificial Sequence
  N-mer
ataggctactggagtgtat

SEQ ID NO: 91 - DNA, 16 bp, Artificial Sequence
  Anchor primer
gatatcgagtcttaag

SEQ ID NO: 92 - DNA, 37 bp, Artificial Sequence
  Ligation product
gatatcgagtcttaagtacacacgaataaaagataac

SEQ ID NO: 93 - DNA, 37 bp, Artificial Sequence
  Ligation product
gatatcgagtcttaagacttttcactggagttgtccc

SEQ ID NO: 94 - DNA, 37 bp, Artificial Sequence
  Ligation product
gatatcgagtcttaagcgatgttaatgggcaaaaatt

SEQ ID NO: 95 - DNA, 37 bp, Artificial Sequence
  Ligation product
gatatcgagtcttaagaggtgatgcaacatacggaaa

SEQ ID NO: 96 - DNA, 16 bp, Artificial Sequence
  Short reverse complementary oligonucleotide
ctatagctcagaattc

SEQ ID NO: 97 - DNA, 42 bp, Artificial Sequence
  Released ligation product
acttttcactggagttgtcccaattcttgttgaattagatgg

SEQ ID NO: 98 - DNA, 41 bp, Artificial Sequence
  Released ligation product
aggtgatgcaacatacggaaaacttacccttaaatttattt

SEQ ID NO: 99 - DNA, 100 bp, Artificial Sequence
  Ligation product
gatatcgagtcttaagtacacacgaataaaagataacaaagatgagtaaaggagaagaacttttcactggagttgtcccaattcttgttgaattagatgg

SEQ ID NO: 100 - DNA, 99 bp, Artificial Sequence
  Ligation product
gatatcgagtcttaagcgatgttaatgggcaaaaattctctgtcagtggagagggtgaaggtgatgcaacatacggaaaacttacccttaaatttattt

SEQ ID NO: 101 - DNA, 83 bp, Artificial Sequence
  Released ligation product
cgatgttaatgggcaaaaattctctgtcagtggagagggtgaaggtgatgcaacatacggaaaacttacccttaaatttattt

SEQ ID NO: 102 - DNA, 153 bp, Artificial Sequence
  Ligation product
gatatcgagtcttaagtacacacgaataaaagataacaaagatgagtaaaggagaagaacttttcactggagttgtcccaattcttgttgaattagatggcgatgttaatgggcaaaaattctctgtcagtggagagggtgaaggtgatgcaa

SEQ ID NO: 103 - DNA, 167 bp, Artificial Sequence
  Released ligation product
tacacacgaataaaagataacaaagatgagtaaaggagaagaacttttcactggagttgtcccaattcttgttgaattagatggcgatgttaatgggcaaaaattctctgtcagtggagagggtgaaggtgatgcaacatacggaaaacttacccttaaatttattt

SEQ ID NO: 104 - DNA, 22 bp, Artificial Sequence
  DNA spacer sequence
ccatggactcatatgccgtgaa